European Patent Application EP 4 556 575 A2, published May 21, 2025. Title: A Method for Sequencing Nucleic Acids. Applicant: Bruker Spatial Biology, Inc. Application EP divisional of EP17812161.2, filed November 21, 2017. The sequence listing filed with the application follows.

SEQUENCE LISTING (99 sequences)

SEQ ID NO: 1 - DNA, 38 bp, Homo sapiens
  source 1..38: mol_type = genomic DNA
accgtgacatgagaagaacaggtcgacataggtcatac

SEQ ID NO: 2 - DNA, 10 bp, synthetic construct
  misc_feature 1..10: note = Example Consensus
  source 1..10: mol_type = other DNA
aacaccacct

SEQ ID NO: 3 - DNA, 24 bp, Homo sapiens
  source 1..24: mol_type = genomic DNA
gtctagctacagtgaaatctcgat

SEQ ID NO: 4 - DNA, 23 bp, Homo sapiens
  source 1..23: mol_type = genomic DNA
tcaaagtgctgggctccggtgcg

SEQ ID NO: 5 - DNA, 27 bp, Homo sapiens
  source 1..27: mol_type = genomic DNA
tagttggagctggtggcgtaggcaaga

SEQ ID NO: 6 - DNA, 23 bp, Homo sapiens
  source 1..23: mol_type = genomic DNA
gaatgatgcacatcatggtggct

SEQ ID NO: 7 - DNA, 23 bp, Homo sapiens
  source 1..23: mol_type = genomic DNA
gcagctcatcacgcagctcatgc

SEQ ID NO: 8 - DNA, 23 bp, Homo sapiens
  source 1..23: mol_type = genomic DNA
atacagctggacaagaagagtac

SEQ ID NO: 9 - DNA, 25 bp, Homo sapiens
  source 1..25: mol_type = genomic DNA
tggctcgagatatcatgagtgattc

SEQ ID NO: 10 - DNA, 23 bp, Homo sapiens
  source 1..23: mol_type = genomic DNA
tcatcataggtcgtcatgcttat

SEQ ID NO: 11 - DNA, 23 bp, Homo sapiens
  source 1..23: mol_type = genomic DNA
atggagtatgtgtctgtggagac

SEQ ID NO: 12 - DNA, 23 bp, Homo sapiens
  source 1..23: mol_type = genomic DNA
gtgcaactctccgtacatcgtgg

SEQ ID NO: 13 - DNA, 23 bp, Homo sapiens
  source 1..23: mol_type = genomic DNA
cagccgcgtgctgcacaccaacg

SEQ ID NO: 14 - RNA, 30 nt, Homo sapiens
  source 1..30: mol_type = unassigned RNA
gcttcagcaccactccactccacattctca

SEQ ID NO: 15 - RNA, 30 nt, Homo sapiens
  source 1..30: mol_type = unassigned RNA
tgtcctcatgtattggtctctcatggcact

SEQ ID NO: 16 - RNA, 30 nt, Homo sapiens
  source 1..30: mol_type = unassigned RNA
ctttcgccaaagtggaggagaccatcgccg

SEQ ID NO: 17 - RNA, 30 nt, Homo sapiens
  source 1..30: mol_type = unassigned RNA
gaaggtgatgtttgggtcaggtgccttagt

SEQ ID NO: 18 - DNA, 50 bp, Homo sapiens
  source 1..50: mol_type = genomic DNA
caaactggtggtggttggagcaggtggtgttgggaaaagcgcactgacaa

SEQ ID NO: 19 - DNA, 12 bp, synthetic construct
  misc_feature 1..12: note = 12-mer attachment position
  source 1..12: mol_type = other DNA
aggacagatgac

SEQ ID NO: 20 - DNA, 12 bp, synthetic construct
  misc_feature 1..12: note = 12-mer attachment position
  source 1..12: mol_type = other DNA
gtatcggatgac

SEQ ID NO: 21 - DNA, 12 bp, synthetic construct
  misc_feature 1..12: note = 12-mer attachment position
  source 1..12: mol_type = other DNA
aggagtgatgac

SEQ ID NO: 22 - DNA, 12 bp, synthetic construct
  misc_feature 1..12: note = 12-mer attachment position
  source 1..12: mol_type = other DNA
aggggtgaggag

SEQ ID NO: 23 - DNA, 12 bp, synthetic construct
  misc_feature 1..12: note = 12-mer attachment position
  source 1..12: mol_type = other DNA
agaggggatgac

SEQ ID NO: 24 - DNA, 12 bp, synthetic construct
  misc_feature 1..12: note = 12-mer attachment position
  source 1..12: mol_type = other DNA
agtggggaggag

SEQ ID NO: 25 - DNA, 12 bp, synthetic construct
  misc_feature 1..12: note = 12-mer attachment position
  source 1..12: mol_type = other DNA
agccgagatgac

SEQ ID NO: 26 - DNA, 12 bp, synthetic construct
  misc_feature 1..12: note = 12-mer attachment position
  source 1..12: mol_type = other DNA
agggtggatgac

SEQ ID NO: 27 - DNA, 12 bp, synthetic construct
  misc_feature 1..12: note = 12-mer attachment position
  source 1..12: mol_type = other DNA
tggatggaaaag

SEQ ID NO: 28 - DNA, 12 bp, synthetic construct
  misc_feature 1..12: note = 12-mer attachment position
  source 1..12: mol_type = other DNA
gaaggagaaaag

SEQ ID NO: 29 - DNA, 12 bp, synthetic construct
  misc_feature 1..12: note = 12-mer attachment position
  source 1..12: mol_type = other DNA
ggggatgaaaag

SEQ ID NO: 30 - DNA, 12 bp, synthetic construct
  misc_feature 1..12: note = 12-mer attachment position
  source 1..12: mol_type = other DNA
gtgagggaaaag

SEQ ID NO: 31 - DNA, 12 bp, synthetic construct
  misc_feature 1..12: note = 12-mer attachment position
  source 1..12: mol_type = other DNA
agccgagaaaag

SEQ ID NO: 32 - DNA, 12 bp, synthetic construct
  misc_feature 1..12: note = 12-mer attachment position
  source 1..12: mol_type = other DNA
cgagaggaaaag

SEQ ID NO: 33 - DNA, 12 bp, synthetic construct
  misc_feature 1..12: note = 12-mer attachment position
  source 1..12: mol_type = other DNA
gagggcgaaaag

SEQ ID NO: 34 - DNA, 12 bp, synthetic construct
  misc_feature 1..12: note = 12-mer attachment position
  source 1..12: mol_type = other DNA
agcgtggaaaag

SEQ ID NO: 35 - DNA, 12 bp, synthetic construct
  misc_feature 1..12: note = 12-mer attachment position
  source 1..12: mol_type = other DNA
tgagaagggtag

SEQ ID NO: 36 - DNA, 12 bp, synthetic construct
  misc_feature 1..12: note = 12-mer attachment position
  source 1..12: mol_type = other DNA
gttgttattgtg

SEQ ID NO: 37 - DNA, 12 bp, synthetic construct
  misc_feature 1..12: note = 12-mer attachment position
  source 1..12: mol_type = other DNA
tttgggtttagg

SEQ ID NO: 38 - DNA, 12 bp, synthetic construct
  misc_feature 1..12: note = 12-mer attachment position
  source 1..12: mol_type = other DNA
gttagtgggaaa

SEQ ID NO: 39 - DNA, 12 bp, synthetic construct
  misc_feature 1..12: note = 12-mer attachment position
  source 1..12: mol_type = other DNA
atgggaaaaagt

SEQ ID NO: 40 - DNA, 12 bp, synthetic construct
  misc_feature 1..12: note = 12-mer attachment position
  source 1..12: mol_type = other DNA
gagttggatgag

SEQ ID NO: 41 - DNA, 12 bp, synthetic construct
  misc_feature 1..12: note = 12-mer attachment position
  source 1..12: mol_type = other DNA
atgttgtgggta

SEQ ID NO: 42 - DNA, 12 bp, synthetic construct
  misc_feature 1..12: note = 12-mer attachment position
  source 1..12: mol_type = other DNA
gagggttttaag

SEQ ID NO: 43 - DNA, 14 bp, synthetic construct
  misc_feature 1..14: note = 14-mer attachment position
  source 1..14: mol_type = other DNA
atcttttccccact

SEQ ID NO: 44 - DNA, 14 bp, synthetic construct
  misc_feature 1..14: note = 14-mer attachment position
  source 1..14: mol_type = other DNA
ccccactatttctt

SEQ ID NO: 45 - DNA, 14 bp, synthetic construct
  misc_feature 1..14: note = 14-mer attachment position
  source 1..14: mol_type = other DNA
ctacccacaacata

SEQ ID NO: 46 - DNA, 14 bp, synthetic construct
  misc_feature 1..14: note = 14-mer attachment position
  source 1..14: mol_type = other DNA
ccatataaacccca

SEQ ID NO: 47 - DNA, 14 bp, synthetic construct
  misc_feature 1..14: note = 14-mer attachment position
  source 1..14: mol_type = other DNA
aaactccaatctcc

SEQ ID NO: 48 - DNA, 14 bp, synthetic construct
  misc_feature 1..14: note = 14-mer attachment position
  source 1..14: mol_type = other DNA
ctattctcaaccta

SEQ ID NO: 49 - DNA, 14 bp, synthetic construct
  misc_feature 1..14: note = 14-mer attachment position
  source 1..14: mol_type = other DNA
ccccctcttttaaa

SEQ ID NO: 50 - DNA, 14 bp, synthetic construct
  misc_feature 1..14: note = 14-mer attachment position
  source 1..14: mol_type = other DNA
ccaatcttacctca

SEQ ID NO: 51 - DNA, 14 bp, synthetic construct
  misc_feature 1..14: note = 14-mer attachment position
  source 1..14: mol_type = other DNA
ccctcacataactt

SEQ ID NO: 52 - DNA, 14 bp, synthetic construct
  misc_feature 1..14: note = 14-mer attachment position
  source 1..14: mol_type = other DNA
ctcctctactttcc

SEQ ID NO: 53 - DNA, 14 bp, synthetic construct
  misc_feature 1..14: note = 14-mer attachment position
  source 1..14: mol_type = other DNA
ccctaaacccaaaa

SEQ ID NO: 54 - DNA, 14 bp, synthetic construct
  misc_feature 1..14: note = 14-mer attachment position
  source 1..14: mol_type = other DNA
cactttttcccatc

SEQ ID NO: 55 - DNA, 14 bp, synthetic construct
  misc_feature 1..14: note = 14-mer attachment position
  source 1..14: mol_type = other DNA
catctgattcctcc

SEQ ID NO: 56 - DNA, 14 bp, synthetic construct
  misc_feature 1..14: note = 14-mer attachment position
  source 1..14: mol_type = other DNA
ctaaaccccctact

SEQ ID NO: 57 - DNA, 14 bp, synthetic construct
  misc_feature 1..14: note = 14-mer attachment position
  source 1..14: mol_type = other DNA
cctttacaaacaca

SEQ ID NO: 58 - DNA, 14 bp, synthetic construct
  misc_feature 1..14: note = 14-mer attachment position
  source 1..14: mol_type = other DNA
ataccaccctcttt

SEQ ID NO: 59 - DNA, 14 bp, synthetic construct
  misc_feature 1..14: note = 14-mer attachment position
  source 1..14: mol_type = other DNA
tattcttctacccc

SEQ ID NO: 60 - DNA, 14 bp, synthetic construct
  misc_feature 1..14: note = 14-mer attachment position
  source 1..14: mol_type = other DNA
tctacccttctcat

SEQ ID NO: 61 - DNA, 14 bp, synthetic construct
  misc_feature 1..14: note = 14-mer attachment position
  source 1..14: mol_type = other DNA
ccacaataacaacc

SEQ ID NO: 62 - DNA, 14 bp, synthetic construct
  misc_feature 1..14: note = 14-mer attachment position
  source 1..14: mol_type = other DNA
accttaacattccc

SEQ ID NO: 63 - DNA, 14 bp, synthetic construct
  misc_feature 1..14: note = 14-mer attachment position
  source 1..14: mol_type = other DNA
atttcccactaacc

SEQ ID NO: 64 - DNA, 14 bp, synthetic construct
  misc_feature 1..14: note = 14-mer attachment position
  source 1..14: mol_type = other DNA
acttaaaaccctcc

SEQ ID NO: 65 - DNA, 14 bp, synthetic construct
  misc_feature 1..14: note = 14-mer attachment position
  source 1..14: mol_type = other DNA
tacctattcctcca

SEQ ID NO: 66 - DNA, 14 bp, synthetic construct
  misc_feature 1..14: note = 14-mer attachment position
  source 1..14: mol_type = other DNA
cccctttctctaag

SEQ ID NO: 67 - DNA, 14 bp, synthetic construct
  misc_feature 1..14: note = 14-mer attachment position
  source 1..14: mol_type = other DNA
gatgatggtaggtg

SEQ ID NO: 68 - DNA, 14 bp, synthetic construct
  misc_feature 1..14: note = 14-mer attachment position
  source 1..14: mol_type = other DNA
atgagaagggtaga

SEQ ID NO: 69 - DNA, 14 bp, synthetic construct
  misc_feature 1..14: note = 14-mer attachment position
  source 1..14: mol_type = other DNA
gttttgttggtgag

SEQ ID NO: 70 - DNA, 14 bp, synthetic construct
  misc_feature 1..14: note = 14-mer attachment position
  source 1..14: mol_type = other DNA
ttagtgtgttggag

SEQ ID NO: 71 - DNA, 14 bp, synthetic construct
  misc_feature 1..14: note = 14-mer attachment position
  source 1..14: mol_type = other DNA
atgtaggagagaga

SEQ ID NO: 72 - DNA, 14 bp, synthetic construct
  misc_feature 1..14: note = 14-mer attachment position
  source 1..14: mol_type = other DNA
gggaatgttaaggt

SEQ ID NO: 73 - DNA, 14 bp, synthetic construct
  misc_feature 1..14: note = 14-mer attachment position
  source 1..14: mol_type = other DNA
ggttagtgggaaat

SEQ ID NO: 74 - DNA, 14 bp, synthetic construct
  misc_feature 1..14: note = 14-mer attachment position
  source 1..14: mol_type = other DNA
ggagggttttaagt

SEQ ID NO: 75 - DNA, 14 bp, synthetic construct
  misc_feature 1..14: note = 14-mer attachment position
  source 1..14: mol_type = other DNA
gtagtgtggatgtt

SEQ ID NO: 76 - DNA, 14 bp, synthetic construct
  misc_feature 1..14: note = 14-mer attachment position
  source 1..14: mol_type = other DNA
cttagagaaagggg

SEQ ID NO: 77 - DNA, 14 bp, synthetic construct
  misc_feature 1..14: note = 14-mer attachment position
  source 1..14: mol_type = other DNA
ggaagaggatgaaa

SEQ ID NO: 78 - DNA, 14 bp, synthetic construct
  misc_feature 1..14: note = 14-mer attachment position
  source 1..14: mol_type = other DNA
aagttatgtgaggg

SEQ ID NO: 79 - DNA, 14 bp, synthetic construct
  misc_feature 1..14: note = 14-mer attachment position
  source 1..14: mol_type = other DNA
ggaaagtagaggag

SEQ ID NO: 80 - DNA, 14 bp, synthetic construct
  misc_feature 1..14: note = 14-mer attachment position
  source 1..14: mol_type = other DNA
ttttgggtttaggg

SEQ ID NO: 81 - DNA, 14 bp, synthetic construct
  misc_feature 1..14: note = 14-mer attachment position
  source 1..14: mol_type = other DNA
agatgtatgggtga

SEQ ID NO: 82 - DNA, 14 bp, synthetic construct
  misc_feature 1..14: note = 14-mer attachment position
  source 1..14: mol_type = other DNA
gatgggaaaaagtg

SEQ ID NO: 83 - DNA, 14 bp, synthetic construct
  misc_feature 1..14: note = 14-mer attachment position
  source 1..14: mol_type = other DNA
ggaggaatcagatg

SEQ ID NO: 84 - DNA, 14 bp, synthetic construct
  misc_feature 1..14: note = 14-mer attachment position
  source 1..14: mol_type = other DNA
agagggattgatga

SEQ ID NO: 85 - DNA, 14 bp, synthetic construct
  misc_feature 1..14: note = 14-mer attachment position
  source 1..14: mol_type = other DNA
tgtgtttgtaaagg

SEQ ID NO: 86 - DNA, 14 bp, synthetic construct
  misc_feature 1..14: note = 14-mer attachment position
  source 1..14: mol_type = other DNA
aaggagtgatagga

SEQ ID NO: 87 - DNA, 14 bp, synthetic construct
  misc_feature 1..14: note = 14-mer attachment position
  source 1..14: mol_type = other DNA
tggtgatttagagg

SEQ ID NO: 88 - DNA, 14 bp, synthetic construct
  misc_feature 1..14: note = 14-mer attachment position
  source 1..14: mol_type = other DNA
ggggtagaagaata

SEQ ID NO: 89 - DNA, 14 bp, synthetic construct
  misc_feature 1..14: note = 14-mer attachment position
  source 1..14: mol_type = other DNA
aagaaatagtgggg

SEQ ID NO: 90 - DNA, 14 bp, synthetic construct
  misc_feature 1..14: note = 14-mer attachment position
  source 1..14: mol_type = other DNA
tatgttgtgggtag

SEQ ID NO: 91 - DNA, 14 bp, synthetic construct
  misc_feature 1..14: note = 14-mer attachment position
  source 1..14: mol_type = other DNA
gttaaagggaggtt

SEQ ID NO: 92 - DNA, 14 bp, synthetic construct
  misc_feature 1..14: note = 14-mer attachment position
  source 1..14: mol_type = other DNA
tggggtttatatgg

SEQ ID NO: 93 - DNA, 14 bp, synthetic construct
  misc_feature 1..14: note = 14-mer attachment position
  source 1..14: mol_type = other DNA
agggaatatggaga

SEQ ID NO: 94 - DNA, 14 bp, synthetic construct
  misc_feature 1..14: note = 14-mer attachment position
  source 1..14: mol_type = other DNA
taggttgagaatag

SEQ ID NO: 95 - DNA, 14 bp, synthetic construct
  misc_feature 1..14: note = 14-mer attachment position
  source 1..14: mol_type = other DNA
tttaaaagaggggg

SEQ ID NO: 96 - DNA, 14 bp, synthetic construct
  misc_feature 1..14: note = 14-mer attachment position
  source 1..14: mol_type = other DNA
tgaggtaagattgg

SEQ ID NO: 97 - DNA, 10 bp, synthetic construct
  misc_feature 1..10: note = Target binding domain
  source 1..10: mol_type = other DNA
agcttcttat

SEQ ID NO: 98 - DNA, 50 bp, synthetic construct
  misc_feature 1..50: note = Target nucleic acid
  source 1..50: mol_type = other DNA
gagactagcagaataggaggataagaagctcgaagagtgaggacaaatgg

SEQ ID NO: 99 - DNA, 10 bp, synthetic construct
  misc_feature 1..10: note = Target binding domain
  source 1..10: mol_type = other DNA
ttcactgtag